European Patent Specification EP 4 441 243 B1, published April 8, 2026. Title: Fixation d'acide nucléique sur une électrode de platine. Applicant: UNIVERSITE PARIS-SACLAY. The sequence listing filed with the application follows.

SEQUENCE LISTING (7 sequences)

SEQ ID NO: 1 - DNA, 26 bp, synthetic construct
  misc_feature 1..26: note = ADN sonde - gene E
  source 1..26: mol_type = other DNA
tcgctattaagtattaacgtacctgt

SEQ ID NO: 2 - DNA, 19 bp, synthetic construct
  misc_feature 1..19: note = ADN sonde - gene N
  source 1..19: mol_type = other DNA
gattgcgggtgccaatgtg

SEQ ID NO: 3 - DNA, 22 bp, synthetic construct
  misc_feature 1..22: note = ADN sonde - gene RdRP
  source 1..22: mol_type = other DNA
ccgccacacatgaccatctcac

SEQ ID NO: 4 - RNA, 26 nt, synthetic construct
  misc_feature 1..26: note = ARN cible - gene E
  source 1..26: mol_type = other RNA
acaggtacgttaatacttaatagcgt

SEQ ID NO: 5 - RNA, 19 nt, synthetic construct
  misc_feature 1..19: note = ARN cible - gene N
  source 1..19: mol_type = other RNA
cacattggcacccgcaatc

SEQ ID NO: 6 - RNA, 22 nt, synthetic construct
  misc_feature 1..22: note = ARN cible - gene RdRP
  source 1..22: mol_type = other RNA
gtgagatggtcatgtgtggcgg

SEQ ID NO: 7 - DNA, 26 bp, synthetic construct
  misc_feature 1..26: note = ADN cible - poly(A)
  source 1..26: mol_type = other DNA
aaaaaaaaaaaaaaaaaaaaaaaaaa